European Patent Application EP 4 506 451 A1, published February 12, 2025. Title: 一种ω-转氨酶突变体及其应用. Applicant: 浙江永太科技股份有限公司. The sequence listing filed with the application follows.

SEQUENCE LISTING (8 sequences)

SEQ ID NO: 1 - DNA, 969 bp, Aspergillus lentulus
  source 1..969: mol_type = genomic DNA
atggcaacaatggataaagtgtttgcaggttattatgcacgtcagaaactgctggaacgtagcgataacccgtttagcaaaggcatcgcatacgttgaaggtaaatttgtgctgcctagcgaagcccgtatccctctgctggatgaaggttttatgggcagcgatctgacctatgatggctttcatgtgtgggatggccgtttttttcgtctggatgatcatctgcagcgtctgctggaaagctgtgataaaatgcgcctgaaatttcctctggcactgagctctgtgaaaaagatcctggtggaaatggtggcgaaaagcggtatccgtgatgcaatgggtaaaatcatcgtgacccgcggtctgacaggtgtgcagggtagcaaacctgaagatctgtataacaacaacatctatctgctggtgctgccgtatatctggctgatggcacctgaaaaacagcgtcatggtggctctgctatcatcacacgtaccgttcgtcgcacacctcctggtgcatttgatcctacaatcaaaaacctgcagtggggcgatctgatccgtggtatgtttgaagccaaagatcgtggcgccacctatccttttctgacagatggtgatacccatctgaccgaaggccctggttttaacatcgtgctggttaaaaacggtatcctgtatacccctgatcgtggtgttctggaaggtattacccgtaaaagcgtgatcgaagtggcgcgtgcaaatagtatcgatgtccgtctggaagtggtgcctgttgaaacagcatatcatgccgatgaaatctttatgtgcaccaccggtggcggtattatgcctattaccctgctggatggcaaaccggttaacgatggtcaggttggtccgattaccaaaaagatctgggatggctattgggaaatgcattataacgcagcatatagctttcctgtggattatggtagcgat

SEQ ID NO: 2 - protein, 323 aa, Aspergillus lentulus
MATMDKVFAGYYARQKLLERSDNPFSKGIAYVEGKFVLPSEARIPLLDEGFMGSDLTYDGFHVWDGRFFRLDDHLQRLLESCDKMRLKFPLALSSVKKILVEMVAKSGIRDAMGKIIVTRGLTGVQGSKPEDLYNNNIYLLVLPYIWLMAPEKQRHGGSAIITRTVRRTPPGAFDPTIKNLQWGDLIRGMFEAKDRGATYPFLTDGDTHLTEGPGFNIVLVKNGILYTPDRGVLEGITRKSVIEVARANSIDVRLEVVPVETAYHADEIFMCTTGGGIMPITLLDGKPVNDGQVGPITKKIWDGYWEMHYNAAYSFPVDYGSD

SEQ ID NO: 3 - DNA, 969 bp, unidentified
  source 1..969: mol_type = genomic DNA
atggcaacaatggataaagtgtttgcaggttattatgcacgtcagaaactgctggaacgtagcgataacccgtttagcaaaggcatcgcatacgttgaaggtaaatttgtgctgcctagcgaagcccgtatccctctgctggatgaaggttttatgggcagcgatctgacctatgatggctttcatgtgtgggatggccgtttttttcgtctggatgatcatctgcagcgtctgctggaaagctgtgataaaatgcgcctgaaatttcctctggcactgagctctgtgaaaaagatcctggtggaaatggtggcgaaaagcggtatccgtgatgcaatgggtaaaatcatcgtgacccgcggtctgacaggtgtgcagggtagcaaacctgaagatctgtataacaacaacatctatctgctggtgctgccgtatatctggctgatggcacctgaaaaacagcgtcatggtggctctgctatcatcacacgtaccgttcgtcgcacacctcctggtgcatttgatcctacaatcaaaaacctgcagtggggcgatctgatccgtggtatgtttgaagccaaagatcgtggcgccacctatccttttctgacagatggtgatacccatctgaccgaaggccctggttttaacatcgtgctggttaaaaacggtatcctgtatacccctgatcgtggtgttctggaaggtattacccgtaaaagcgtgatcgaagtggcgcgtgcaaatagtatcgatgtccgtctggaagtggtgcctgttgaaacagcatatcatgccgatgaaatctttatgtgcaccaccgccggcggtattatgcctattaccctgctggatggcaaaccggttaacgatggtcaggttggtccgattaccaaaaagatctgggatggctattgggaaatgcattataacgcagcatatagctttcctgtggattatggtagcgat

SEQ ID NO: 4 - protein, 323 aa, unidentified
MATMDKVFAGYYARQKLLERSDNPFSKGIAYVEGKFVLPSEARIPLLDEGFMGSDLTYDGFHVWDGRFFRLDDHLQRLLESCDKMRLKFPLALSSVKKILVEMVAKSGIRDAMGKIIVTRGLTGVQGSKPEDLYNNNIYLLVLPYIWLMAPEKQRHGGSAIITRTVRRTPPGAFDPTIKNLQWGDLIRGMFEAKDRGATYPFLTDGDTHLTEGPGFNIVLVKNGILYTPDRGVLEGITRKSVIEVARANSIDVRLEVVPVETAYHADEIFMCTTAGGIMPITLLDGKPVNDGQVGPITKKIWDGYWEMHYNAAYSFPVDYGSD

SEQ ID NO: 5 - DNA, 969 bp, unidentified
  source 1..969: mol_type = genomic DNA
atggcaacaatggataaagtgtttgcaggttattatgcacgtcagaaactgctggaacgtagcgataacccgtttagcaaaggcatcgcatacgttgaaggtaaatttgtgctgcctagcgaagcccgtatccctctgctggatgaaggttttatgggcagcgatctgacctatgatggctttcatgtgtgggatggccgtttttttcgtctggatgatcatctgcagcgtctgctggaaagctgtgataaaatgcgcctgaaatttcctctggcactgagctctgtgaaaaagatcctggtggaaatggtggcgaaaagcggtatccgtgatgcaatgggtatgatcatcgtgacccgcggtctgacaggtgtgcagggtagcaaacctgaagatctgtataacaacaacatctatctgctggtgctgccgtatatctggctgatggcacctgaaaaacagcgtcatggtggctctgctatcatcacacgtaccgttcgtcgcacacctcctggtgcatttgatcctacaatcaaaaacctgcagtggggcgatctgatccgtggtatgtttgaagccaaagatcgtggcgccacctatccttttctgacagatggtgatacccatctgaccgaaggccctggttttaacatcgtgctggttaaaaacggtatcctgtatacccctgatcgtggtgttctggaaggtattacccgtaaaagcgtgatcgaagtggcgcgtgcaaatagtatcgatgtccgtctggaagtggtgcctgttgaaacagcatatcatgccgatgaaatctttatgtgcaccaccggtggcggtattatgcctattaccctgctggatggcaaaccggttaacgatggtcaggttggtccgattaccaaaaagatctgggatggctattgggaaatgcattataacgcagcatatagctttcctgtggattatggtagcgat

SEQ ID NO: 6 - protein, 323 aa, unidentified
MATMDKVFAGYYARQKLLERSDNPFSKGIAYVEGKFVLPSEARIPLLDEGFMGSDLTYDGFHVWDGRFFRLDDHLQRLLESCDKMRLKFPLALSSVKKILVEMVAKSGIRDAMGMIIVTRGLTGVQGSKPEDLYNNNIYLLVLPYIWLMAPEKQRHGGSAIITRTVRRTPPGAFDPTIKNLQWGDLIRGMFEAKDRGATYPFLTDGDTHLTEGPGFNIVLVKNGILYTPDRGVLEGITRKSVIEVARANSIDVRLEVVPVETAYHADEIFMCTTGGGIMPITLLDGKPVNDGQVGPITKKIWDGYWEMHYNAAYSFPVDYGSD

SEQ ID NO: 7 - DNA, 969 bp, unidentified
  source 1..969: mol_type = genomic DNA
atggcaacaatggataaagtgtttgcaggttattatgcacgtcagaaactgctggaacgtagcgataacccgtttagcaaaggcatcgcatacgttgaaggtaaatttgtgctgcctagcgaagcccgtatccctctgctggatgaaggttttatgggcagcgatctgacctatgatggctttcatgtgtgggatggccgtttttttcgtctggatgatcatctgcagcgtctgctggaaagctgtgataaaatgcgcctgaaatttcctctggcactgagctctgtgcgcaagatcctggtggaaatggtggcgaaaagcggtatccgtgatgcaatgggtatgatcatcgtgacccgcggtctgacaggtgtgcagggtagcaaacctgaagatctgtataacaacaacatctatctgctggtgctgccgtatatctggctgatggcacctgaaaaacagcgtcatggtggctctgctatcatcacacgtaccgttcgtcgcacacctcctggtgcatttgatcctacaatcaaaaacctgcagtggggcgatctgatccgtggtatgtttgaagccaaagatcgtggcgccacctatccttttctgacagatggtgatacccatctgaccgaaggccctggttttaacatcgtgctggttaaaaacggtatcctgtatacccctgatcgtggtgttctggaaggtattacccgtaaaagcgtgatcgaagtggcgcgtgcaaatagtatcgatgtccgtctggaagtggtgcctgttgaaacagcatatcatgccgatgaaatctttatgtgcaccaccggtggcggtattatgcctattaccctgctggatggcaaaccggttaacgatggtcaggttggtccgattaccaaaaagatctgggatggctattgggaaatgcattataacgcagcatatagctttcctgtggattatggtagcgat

SEQ ID NO: 8 - protein, 323 aa, unidentified
MATMDKVFAGYYARQKLLERSDNPFSKGIAYVEGKFVLPSEARIPLLDEGFMGSDLTYDGFHVWDGRFFRLDDHLQRLLESCDKMRLKFPLALSSVRKILVEMVAKSGIRDAMGMIIVTRGLTGVQGSKPEDLYNNNIYLLVLPYIWLMAPEKQRHGGSAIITRTVRRTPPGAFDPTIKNLQWGDLIRGMFEAKDRGATYPFLTDGDTHLTEGPGFNIVLVKNGILYTPDRGVLEGITRKSVIEVARANSIDVRLEVVPVETAYHADEIFMCTTGGGIMPITLLDGKPVNDGQVGPITKKIWDGYWEMHYNAAYSFPVDYGSD